European Patent Application EP 4 537 907 A1, published April 16, 2025. Title: CD248 INHIBITORS AND USES THEREOF. Applicant: Enthera S.r.l. The sequence listing filed with the application follows.

SEQUENCE LISTING (153 sequences)

SEQ ID NO: 1 - protein, 5 aa, synthetic construct
SYAMS

SEQ ID NO: 2 - protein, 7 aa, synthetic construct
SGGYYWS

SEQ ID NO: 3 - protein, 5 aa, synthetic construct
SYAMH

SEQ ID NO: 4 - protein, 17 aa, synthetic construct
AISGSGGSTYYADSVKG

SEQ ID NO: 5 - protein, 16 aa, synthetic construct
YIYYSGSTYYNPSLKS

SEQ ID NO: 6 - protein, 17 aa, synthetic construct
VISYDGSNKYYADSVKG

SEQ ID NO: 7 - protein, 5 aa, synthetic construct
LTGTT

SEQ ID NO: 8 - protein, 11 aa, synthetic construct
VRGRSATYFDY

SEQ ID NO: 9 - protein, 7 aa, synthetic construct
RSGGFDY

SEQ ID NO: 10 - protein, 12 aa, synthetic construct
SIAAAGTRWFDP

SEQ ID NO: 11 - protein, 12 aa, synthetic construct
NNHPRGERLPQY

SEQ ID NO: 12 - protein, 14 aa, synthetic construct
TKARWFGVTTYMDV

SEQ ID NO: 13 - protein, 17 aa, synthetic construct
KSSRSVLYSSNNKNYLA

SEQ ID NO: 14 - protein, 14 aa, synthetic construct
TGSSSNIGAGYDVR

SEQ ID NO: 15 - protein, 16 aa, synthetic construct
RSSQSLLHSNGYNYLD

SEQ ID NO: 16 - protein, 11 aa, synthetic construct
RASQGISSWLA

SEQ ID NO: 17 - protein, 11 aa, synthetic construct
RASQSVGSYLN

SEQ ID NO: 18 - protein, 17 aa, synthetic construct
KSSQSVLYSSNNKNYLA

SEQ ID NO: 19 - protein, 7 aa, synthetic construct
WASTRES

SEQ ID NO: 20 - protein, 7 aa, synthetic construct
ANNNRPS

SEQ ID NO: 21 - protein, 7 aa, synthetic construct
FTSNRAS

SEQ ID NO: 22 - protein, 7 aa, synthetic construct
AASSLQS

SEQ ID NO: 23 - protein, 7 aa, synthetic construct
VASRLQS

SEQ ID NO: 24 - protein, 9 aa, synthetic construct
QQYYSTPYS

SEQ ID NO: 25 - protein, 11 aa, synthetic construct
QSYDISLSGSL

SEQ ID NO: 26 - protein, 9 aa, synthetic construct
MQSIQLPRT

SEQ ID NO: 27 - protein, 9 aa, synthetic construct
QQANSFPLT

SEQ ID NO: 28 - protein, 9 aa, synthetic construct
QQSYSTPLT

SEQ ID NO: 29 - protein, 9 aa, synthetic construct
QQYYSTPPT

SEQ ID NO: 30 - protein, 114 aa, synthetic construct
EVQLLESGGGLVQPGGSLRLSCAASGFTFSSYAMSWVRQAPGKGLEWVSAISGSGGSTYYADSVKGRFTISRDNSKNTLYLQMNSLRAEDTAVYYCAKLTGTTWGQGTLVTVSS

SEQ ID NO: 31 - protein, 121 aa, synthetic construct
QVQLVESGPGLVKPSQTLSLTCTVSGGSISSGGYYWSWIRQHPGKGLEWIGYIYYSGSTYYNPSLKSRVTISVDTSKNQFSLKLSSVTAADTAVYYCARVRGRSATYFDYWGQGTTVTVSS

SEQ ID NO: 32 - protein, 116 aa, synthetic construct
EVQLLESGGGLVQPGGSLRLSCAASGFTFSSYAMSWVRQAPGKGLEWVSAISGSGGSTYYADSVKGRFTISRDNSKNTLYLQMNSLRAEDTAVYYCAARSGGFDYWGQGTLVTVSS

SEQ ID NO: 33 - protein, 121 aa, synthetic construct
EVQLLESGGGVVQPGRSLRLSCAASGFTFSSYAMHWVRQAPGKGLEWVAVISYDGSNKYYADSVKGRFTISRDNSKNTLYLQMNSLRAEDTAVYYCARSIAAAGTRWFDPWGQGTLVTVSS

SEQ ID NO: 34 - protein, 121 aa, synthetic construct
QVQLQESGGGVVQPGRSLRLSCAASGFTFSSYAMHWVRQAPGKGLEWVAVISYDGSNKYYADSVKGRFTISRDNSKNTLYLQMNSLRAEDTAVYYCARNNHPRGERLPQYWGQGTLVTVSS

SEQ ID NO: 35 - protein, 123 aa, synthetic construct
QVQLVQSGGGVVQPGRSLRLSCAASGFTFSSYAMHWVRQAPGKGLEWVAVISYDGSNKYYADSVKGRFTISRDNSKNTLYLQMNSLRAEDTAVYYCARTKARWFGVTTYMDVWGKGTLVTVSS

SEQ ID NO: 36 - protein, 113 aa, synthetic construct
DIVMTQSPDSLAVSLGERATINCKSSRSVLYSSNNKNYLAWYQQKPGQPPKLLIYWASTRESGVPDRFSGSGSGTDFTLTISSLQAEDVAVYYCQQYYSTPYSFGQGTKVEIK

SEQ ID NO: 37 - protein, 111 aa, synthetic construct
QSVLTQPPSVSGAPGQRVTISCTGSSSNIGAGYDVRWYQQLPGTAPKLLIYANNNRPSGVPDRFSGSKSGTSASLAITGLQTEDEADYYCQSYDISLSGSLFGGGTKLTVL

SEQ ID NO: 38 - protein, 112 aa, synthetic construct
DVVMTQSPLSLPVTPGEPASISCRSSQSLLHSNGYNYLDWYVQKPGQSPQRLIYFTSNRASGVPDRFSGSGSGTDFTLKISRVEAEDVGVYYCMQSIQLPRTFGQGTKVEIK

SEQ ID NO: 39 - protein, 107 aa, synthetic construct
DIQLTQSPSSVSASVGDRVTITCRASQGISSWLAWYQQKPGKAPKLLIYAASSLQSGVPSRFSGSGSGTDFTLTISSLQPEDFATYYCQQANSFPLTFGGGTKLEIK

SEQ ID NO: 40 - protein, 107 aa, synthetic construct
DIQLTQSPSSLSASVGDRVTITCRASQSVGSYLNWYQHKPGKAPKLLIYVASRLQSGVPSRFSGSGSGTDFTLTINSLQPEDFATYYCQQSYSTPLTFGGGTKVEIK

SEQ ID NO: 41 - protein, 113 aa, synthetic construct
DIVMTQSPDSLAVSLGERATINCKSSQSVLYSSNNKNYLAWYQQKPGQPPKLLIYWASTRESGVPDRFSGSGSGTDFTLTISSLQAEDVAVYYCQQYYSTPPTFGQGTKVEIK

SEQ ID NO: 42 - DNA, 342 bp, synthetic construct
  source 1..342: mol_type = other DNA
gaggtacaactgctcgagtcaggcggggggctcgtccaaccagggggatctttgcgcctgtcttgtgctgcttctggttttacattttccagctatgcgatgagctgggtacggcaggccccaggcaaaggactcgagtgggtgtcagcgattagtggtagtggtgggtctacatattacgctgacagcgtgaaggggcggtttacaatttctcgagacaactctaagaacaccctgtaccttcaaatgaacagtctgagagccgaggatactgctgtttattattgcgcgaaacttacgggtacaacttggggacaggggacactcgtcactgtctcttca

SEQ ID NO: 43 - DNA, 363 bp, synthetic construct
  source 1..363: mol_type = other DNA
caggtccaattggtggaaagtgggccgggccttgtcaaaccttctcagacactctctctcacctgtactgtttcaggtggaagcataagtagtggtggttattactggtcatggattcgccaacatcctgggaagggacttgaatggatcggttacatttattattccggttccacctactacaatccgagtctcaagtctcgcgtaacgatatccgttgatacttctaagaatcagttcagtcttaaattgagttcagtcaccgccgccgatacagcggtctattattgtgcaagggtccgaggccggtccgctacatactttgactactggggtcaggggacaaccgtaacagtatcttca

SEQ ID NO: 44 - DNA, 348 bp, synthetic construct
  source 1..348: mol_type = other DNA
gaggtccaacttctcgaaagcggcggtggcctggtgcagccgggtggttcactgcggttgtcctgtgctgcaagcggatttacatttagcagctatgccatgtcatgggtacgacaggcacccggaaagggccttgagtgggtatccgcaatttcaggctcaggcggcagcacctattatgccgatagcgttaagggaagatttaccatcagccgagataattctaaaaatacactttaccttcaaatgaacagtttgcgggctgaggatactgcagtgtattattgcgctgcgcgatctggtgggtttgactattgggggcagggcaccttggtaacagttagttct

SEQ ID NO: 45 - DNA, 363 bp, synthetic construct
  source 1..363: mol_type = other DNA
gaggtacaactcttggaaagcggcggcggtgtagtacagccgggtagaagtctccgactgagctgcgccgcttctggattcacattttcctcctatgcgatgcattgggtcagacaggcccctgggaaagggttggaatgggtagctgttattagttatgatggaagcaataagtattacgcagattccgttaaaggccgattcaccatttcacgagataattcaaagaacactctttatttgcagatgaactcactcagagccgaagatacggcggtgtactactgtgctagaagcattgcggctgcagggacgcgctggttcgatccgtggggtcagggaactctggttacagtaagcagc

SEQ ID NO: 46 - DNA, 363 bp, synthetic construct
  source 1..363: mol_type = other DNA
caggtccaactgcaggagtcaggtggaggcgtcgtacaaccagggcgaagtctgcgactttcatgcgctgcaagcggtttcacattctcctcatacgcgatgcactgggtgcggcaggctcccggcaagggcctggaatgggtcgcggttatctcttacgacggaagcaacaaatactacgccgacagtgtgaagggccgattcacaataagtcgggataattcaaaaaacacattgtacttgcaaatgaacagcctgcgcgcggaggacactgctgtctactactgtgcccgaaataatcatcccagaggtgaacgcttgccgcagtattggggtcagggtacactcgttactgtatcctct

SEQ ID NO: 47 - DNA, 369 bp, synthetic construct
  source 1..369: mol_type = other DNA
caggttcagttggttcaatctggaggcggagtcgtccaacctggtcggtcacttaggctttcttgtgcggcatcaggtttcaccttctcatcttacgcgatgcactgggtacggcaagcgcctggaaaaggtctggagtgggtcgccgtgatttcctacgacgggagtaataaatattatgcagacagtgtcaaaggcaggttcacgatttcaagggacaactctaagaataccttgtaccttcaaatgaactccctgcgagcggaagatacggcggtttattactgtgctcggacgaaagcccgctggtttggagtgaccacgtatatggacgtttgggggaaaggtactcttgtgactgtctcttct

SEQ ID NO: 48 - DNA, 339 bp, synthetic construct
  source 1..339: mol_type = other DNA
gatatagtaatgacacaatcacctgacagcctcgcagttagcctcggagagcgggcgaccattaactgcaagagcagtcggtcagttctctactcaagtaacaataagaactacctcgcatggtaccaacaaaagcccggccaacccccaaagttgctcatatactgggcatctacccgggaaagcggggtgccggatcgcttttccggcagcggtagcggcactgacttcaccctcacgatttcttctcttcaggcagaggacgtagcggtatattactgtcagcagtattatagcactccttattctttcgggcaggggaccaaagtggaaattaag

SEQ ID NO: 49 - DNA, 333 bp, synthetic construct
  source 1..333: mol_type = other DNA
caatctgtcttgactcagcctcccagtgtttctggagcgccgggccagagggtgactattagttgcaccggaagttcaagtaatataggtgcgggttatgacgttcgatggtatcagcagctccccggaactgcgcctaagctccttatatacgcaaataacaacaggcccagtggggtaccagatcggttctctgggtctaaaagcggcacatccgcgagccttgcaatcacagggttgcaaactgaagatgaagctgactattattgccaaagctacgacataagtcttagcggctccctgttcggcggggggactaaattgaccgttctg

SEQ ID NO: 50 - DNA, 336 bp, synthetic construct
  source 1..336: mol_type = other DNA
gatgttgtaatgactcaatcccctctgagccttcccgttacaccgggggagccagcctcaataagctgccgatcctctcaatctctcctgcatagtaatggctacaattatcttgattggtatgttcagaaaccaggtcagtcacctcaaagactcatctatttcactagcaaccgagccagcggggtaccggaccgattttcaggcagcggctcaggtacagatttcacccttaagattagcagagtggaagccgaggatgttggggtctattactgtatgcaatccatacagctgccgaggacgtttggacaaggaactaaagtggagataaag

SEQ ID NO: 51 - DNA, 321 bp, synthetic construct
  source 1..321: mol_type = other DNA
gatattcagctcacccagtcccctagcagtgtttcagcctctgttggggaccgcgtcacaataacttgtcgcgcgtcacaaggaataagctcatggctggcctggtatcaacaaaagccaggtaaagctcccaaacttcttatatatgccgcgtcatctctccagagcggggttccttcccgattttccggttccggttcaggcacggacttcacattgacgattagttccttgcaacccgaagattttgcaacatattactgtcaacaagcgaatagctttccgctgacattcggtggtggcacgaaattggagattaaa

SEQ ID NO: 52 - DNA, 321 bp, synthetic construct
  source 1..321: mol_type = other DNA
gatattcagttgacacagagtccctccagtttgagcgcaagtgtaggagacagagttacgataacttgtcgagcctcacaaagtgtcgggtcttacttgaattggtatcagcacaaacccggcaaggcaccgaagctgttgatatatgtggctagtagattgcagagcggggtgccttcaaggttttcagggtccggctctgggactgattttacgttgacaattaatagcctgcaaccggaggatttcgctacatattactgccagcagagctactcaacgccgctcacatttggaggcgggacgaaggttgagattaag

SEQ ID NO: 53 - DNA, 339 bp, synthetic construct
  source 1..339: mol_type = other DNA
gacattgtaatgacacagagtcctgacagtctcgctgtatctctcggagagcgggcgactatcaactgtaaatcttcacaatcagtgctttattcctctaacaacaaaaactaccttgcgtggtatcaacaaaagcctggtcagcctcctaaactgctgatatattgggcgtccactcgcgaatccggcgttcccgaccgatttagcggtagcggatcaggcacggattttaccctcaccatatcatccttgcaggcggaggatgtcgctgtttactattgccagcaatactactcaacccctcccacctttggacaaggaaccaaggtggagataaaa

SEQ ID NO: 54 - protein, 327 aa, synthetic construct
ASTKGPSVFPLAPCSRSTSESTAALGCLVKDYFPEPVTVSWNSGALTSGVHTFPAVLQSSGLYSLSSVVTVPSSSLGTKTYTCNVDHKPSNTKVDKRVESKYGPPCPSCPAPEFLGGPSVFLFPPKPKDTLMISRTPEVTCVVVDVSQEDPEVQFNWYVDGVEVHNAKTKPREEQFNSTYRVVSVLTVLHQDWLNGKEYKCKVSNKGLPSSIEKTISKAKGQPREPQVYTLPPSQEEMTKNQVSLTCLVKGFYPSDIAVEWESNGQPENNYKTTPPVLDSDGSFFLYSRLTVDKSRWQEGNVFSCSVMHEALHNHYTQKSLSLSLGK

SEQ ID NO: 55 - protein, 326 aa, synthetic construct
ASTKGPSVFPLAPCSRSTSESTAALGCLVKDYFPEPVTVSWNSGALTSGVHTFPAVLQSSGLYSLSSVVTVPSSNFGTQTYTCNVDHKPSNTKVDKTVERKCCVECPPCPAPPVAGPSVFLFPPKPKDTLMISRTPEVTCVVVDVSHEDPEVQFNWYVDGVEVHNAKTKPREEQFNSTFRVVSVLTVVHQDWLNGKEYKCKVSNKGLPAPIEKTISKTKGQPREPQVYTLPPSREEMTKNQVSLTCLVKGFYPSDISVEWESNGQPENNYKTTPPMLDSDGSFFLYSKLTVDKSRWQQGNVFSCSVMHEALHNHYTQKSLSLSPGK

SEQ ID NO: 56 - protein, 106 aa, synthetic construct
GQPKANPTVTLFPPSSEELQANKATLVCLISDFYPGAVTVAWKADGSPVKAGVETTKPSKQSNNKYAASSYLSLTPEQWKSHRSYSCQVTHEGSTVEKTVAPTECS

SEQ ID NO: 57 - protein, 106 aa, synthetic construct
GQPKAAPSVTLFPPSSEELQANKATLVCLISDFYPGAVTVAWKADSSPVKAGVETTTPSKQSNNKYAASSYLSLTPEQWKSHRSYSCQVTHEGSTVEKTVAPTECS

SEQ ID NO: 58 - protein, 107 aa, synthetic construct [sequence omitted]

SEQ ID NO: 59 - protein, 13 aa, synthetic construct
LYSSNNKNYLAWY

SEQ ID NO: 60 - protein, 12 aa, synthetic construct
RSVLYSSNNKNY

SEQ ID NO: 61 - protein, 10 aa, synthetic construct
LLIYWASTRE

SEQ ID NO: 62 - protein, 327 aa, synthetic construct
ASTKGPSVFPLAPCSRSTSESTAALGCLVKDYFPEPVTVSWNSGALTSGVHTFPAVLQSSGLYSLSSVVTVPSSSLGTKTYTCNVDHKPSNTKVDKRVESKYGPPCPPCPAPEFEGGPSVFLFPPKPKDTLMISRTPEVTCVVVDVSQEDPEVQFNWYVDGVEVHNAKTKPREEQFNSTYRVVSVLTVLHQDWLNGKEYKCKVSNKGLPSSIEKTISKAKGQPREPQVYTLPPSQEEMTKNQVSLTCLVKGFYPSDIAVEWESNGQPENNYKTTPPVLDSDGSFFLYSRLTVDKSRWQEGNVFSCSVMHEALHNHYTQKSLSLSLGK

SEQ ID NO: 63 - protein, 8 aa, synthetic construct
QQYYSTPY

SEQ ID NO: 64 - protein, 7 aa, synthetic construct
GFTFSSY

SEQ ID NO: 65 - protein, 10 aa, synthetic construct
GFTFSSYAMS

SEQ ID NO: 66 - protein, 6 aa, synthetic construct
SSYAMS

SEQ ID NO: 67 - protein, 8 aa, synthetic construct
GFTFSSYA

SEQ ID NO: 68 - protein, 6 aa, synthetic construct
SGSGGS

SEQ ID NO: 69 - protein, 10 aa, synthetic construct
AISGSGGSTY

SEQ ID NO: 70 - protein, 13 aa, synthetic construct
WVSAISGSGGSTY

SEQ ID NO: 71 - protein, 8 aa, synthetic construct
ISGSGGST

SEQ ID NO: 72 - protein, 6 aa, synthetic construct
AKLTGT

SEQ ID NO: 73 - protein, 7 aa, synthetic construct
AKLTGTT

SEQ ID NO: 74 - protein, 10 aa, synthetic construct
IGAGYDVRWY

SEQ ID NO: 75 - protein, 9 aa, synthetic construct
SSNIGAGYD

SEQ ID NO: 76 - protein, 10 aa, synthetic construct
LLIYANNNRP

SEQ ID NO: 77 - protein, 10 aa, synthetic construct
QSYDISLSGS

SEQ ID NO: 78 - protein, 9 aa, synthetic construct
GGSISSGGY

SEQ ID NO: 79 - protein, 12 aa, synthetic construct
GGSISSGGYYWS

SEQ ID NO: 80 - protein, 15 aa, synthetic construct
WYQHKPGKAPKLLIY

SEQ ID NO: 81 - protein, 32 aa, synthetic construct
GVPDRFSGSGSGTDFTLTISSLQAEDVAVYYC

SEQ ID NO: 82 - protein, 32 aa, synthetic construct
GVPDRFSGSKSGTSASLAITGLQTEDEADYYC

SEQ ID NO: 83 - protein, 32 aa, synthetic construct
GVPDRFSGSGSGTDFTLKISRVEAEDVGVYYC

SEQ ID NO: 84 - protein, 32 aa, synthetic construct
GVPSRFSGSGSGTDFTLTISSLQPEDFATYYC

SEQ ID NO: 85 - protein, 32 aa, synthetic construct
GVPSRFSGSGSGTDFTLTINSLQPEDFATYYC

SEQ ID NO: 86 - protein, 32 aa, synthetic construct; identical to SEQ ID NO: 81

SEQ ID NO: 87 - protein, 10 aa, synthetic construct
FGQGTKVEIK

SEQ ID NO: 88 - protein, 8 aa, synthetic construct
SSGGYYWS

SEQ ID NO: 89 - protein, 10 aa, synthetic construct
GGSISSGGYY

SEQ ID NO: 90 - protein, 5 aa, synthetic construct
YYSGS

SEQ ID NO: 91 - protein, 9 aa, synthetic construct
YIYYSGSTY

SEQ ID NO: 92 - protein, 12 aa, synthetic construct
WIGYIYYSGSTY

SEQ ID NO: 93 - protein, 7 aa, synthetic construct
IYYSGST

SEQ ID NO: 94 - protein, 12 aa, synthetic construct
ARVRGRSATYFD

SEQ ID NO: 95 - protein, 13 aa, synthetic construct
ARVRGRSATYFDY

SEQ ID NO: 96 - protein, 12 aa, synthetic construct
LHSNGYNYLDWY

SEQ ID NO: 97 - protein, 11 aa, synthetic construct
QSLLHSNGYNY

SEQ ID NO: 98 - protein, 10 aa, synthetic construct
RLIYFTSNRA

SEQ ID NO: 99 - protein, 10 aa, synthetic construct
FGGGTKLTVL

SEQ ID NO: 100 - protein, 8 aa, synthetic construct
MQSIQLPR

SEQ ID NO: 101 - protein, 8 aa, synthetic construct
AARSGGFD

SEQ ID NO: 102 - protein, 9 aa, synthetic construct
AARSGGFDY

SEQ ID NO: 103 - protein, 7 aa, synthetic construct
SSWLAWY

SEQ ID NO: 104 - protein, 6 aa, synthetic construct
QGISSW

SEQ ID NO: 105 - protein, 10 aa, synthetic construct
LLIYAASSLQ

SEQ ID NO: 106 - protein, 10 aa, synthetic construct
FGGGTKLEIK

SEQ ID NO: 107 - protein, 8 aa, synthetic construct
QQANSFPL

SEQ ID NO: 108 - protein, 7 aa, synthetic construct
GFTFSSY

SEQ ID NO: 109 - protein, 10 aa, synthetic construct
GFTFSSYAMH

SEQ ID NO: 110 - protein, 6 aa, synthetic construct
SSYAMH

SEQ ID NO: 111 - protein, 8 aa, synthetic construct
GFTFSSYA

SEQ ID NO: 112 - protein, 6 aa, synthetic construct
SYDGSN

SEQ ID NO: 113 - protein, 10 aa, synthetic construct
VISYDGSNKY

SEQ ID NO: 114 - protein, 13 aa, synthetic construct
WVAVISYDGSNKY

SEQ ID NO: 115 - protein, 8 aa, synthetic construct
ISYDGSNK

SEQ ID NO: 116 - protein, 13 aa, synthetic construct
ARSIAAAGTRWFD

SEQ ID NO: 117 - protein, 14 aa, synthetic construct
ARSIAAAGTRWFDP

SEQ ID NO: 118 - protein, 7 aa, synthetic construct
GSYLNWY

SEQ ID NO: 119 - protein, 6 aa, synthetic construct
QSVGSY

SEQ ID NO: 120 - protein, 10 aa, synthetic construct
LLIYVASRLQ

SEQ ID NO: 121 - protein, 10 aa, synthetic construct
FGGGTKVEIK

SEQ ID NO: 122 - protein, 8 aa, synthetic construct
QQSYSTPL

SEQ ID NO: 123 - protein, 13 aa, synthetic construct
ARNNHPRGERLPQ

SEQ ID NO: 124 - protein, 14 aa, synthetic construct
ARNNHPRGERLPQY

SEQ ID NO: 125 - protein, 13 aa, synthetic construct
LYSSNNKNYLAWY

SEQ ID NO: 126 - protein, 12 aa, synthetic construct
QSVLYSSNNKNY

SEQ ID NO: 127 - protein, 8 aa, synthetic construct
QQYYSTPP

SEQ ID NO: 128 - protein, 15 aa, synthetic construct
ARTKARWFGVTTYMD

SEQ ID NO: 129 - protein, 16 aa, synthetic construct
ARTKARWFGVTTYMDV

SEQ ID NO: 130 - protein, 30 aa, synthetic construct
EVQLLESGGGLVQPGGSLRLSCAASGFTFS

SEQ ID NO: 131 - protein, 30 aa, synthetic construct
QVQLVESGPGLVKPSQTLSLTCTVSGGSIS

SEQ ID NO: 132 - protein, 30 aa, synthetic construct
EVQLLESGGGVVQPGRSLRLSCAASGFTFS

SEQ ID NO: 133 - protein, 30 aa, synthetic construct
QVQLQESGGGVVQPGRSLRLSCAASGFTFS

SEQ ID NO: 134 - protein, 30 aa, synthetic construct
QVQLVQSGGGVVQPGRSLRLSCAASGFTFS

SEQ ID NO: 135 - protein, 14 aa, synthetic construct
WVRQAPGKGLEWVS

SEQ ID NO: 136 - protein, 14 aa, synthetic construct
WIRQHPGKGLEWIG

SEQ ID NO: 137 - protein, 14 aa, synthetic construct
WVRQAPGKGLEWVA

SEQ ID NO: 138 - protein, 32 aa, synthetic construct
RFTISRDNSKNTLYLQMNSLRAEDTAVYYCAK

SEQ ID NO: 139 - protein, 32 aa, synthetic construct
RVTISVDTSKNQFSLKLSSVTAADTAVYYCAR

SEQ ID NO: 140 - protein, 11 aa, synthetic construct
WGQGTLVTVSS

SEQ ID NO: 141 - protein, 11 aa, synthetic construct
WGQGTTVTVSS

SEQ ID NO: 142 - protein, 11 aa, synthetic construct
WGKGTLVTVSS

SEQ ID NO: 143 - protein, 23 aa, synthetic construct
DIVMTQSPDSLAVSLGERATINC

SEQ ID NO: 144 - protein, 22 aa, synthetic construct
QSVLTQPPSVSGAPGQRVTISC

SEQ ID NO: 145 - protein, 23 aa, synthetic construct
DVVMTQSPLSLPVTPGEPASISC

SEQ ID NO: 146 - protein, 23 aa, synthetic construct
DIQLTQSPSSVSASVGDRVTITC

SEQ ID NO: 147 - protein, 23 aa, synthetic construct
DIQLTQSPSSLSASVGDRVTITC

SEQ ID NO: 148 - protein, 15 aa, synthetic construct
WYQQKPGQPPKLLIY

SEQ ID NO: 149 - protein, 15 aa, synthetic construct
WYQQLPGTAPKLLIY

SEQ ID NO: 150 - protein, 15 aa, synthetic construct
WYVQKPGQSPQRLIY

SEQ ID NO: 151 - protein, 15 aa, synthetic construct
WYQQKPGKAPKLLIY

SEQ ID NO: 152 - protein, 32 aa, synthetic construct
RFTISRDNSKNTLYLQMNSLRAEDTAVYYCAA

SEQ ID NO: 153 - protein, 32 aa, synthetic construct
RFTISRDNSKNTLYLQMNSLRAEDTAVYYCAR